European Patent Specification EP 3 356 809 B1, published May 8, 2024. Title: Dual Mediator Biosensor. Applicant: The Bio Nano Centre Limited. Application EP16794388.5. The sequence listing filed with the application follows.

SEQUENCE LISTING (8 sequences)

SEQ ID NO: 1 - protein, 175 aa, Rhizobium sp. NT-26
MSRCQNMVDIGRRQFLRGGALAAAGATAAVFGVGAPQARAATAAAGVEYPANRLANISELTLNEPLDVAYPDEDAAGVLLKLGTRVEGGVGPDGDIVGFSTICPHKGFPLSYSADNKTFNCPGHFSVFDPEKGGQQVWGQATQNLPQYVLRVADNGDIFAEGVDELIYGRLSNVL

SEQ ID NO: 2 - protein, 40 aa, Rhizobium sp. NT-26
MSRCQNMVDIGRRQFLRGGALAAAGATAAVFGVGAPQARA

SEQ ID NO: 3 - protein, 150 aa, Rhizobium sp. NT-26
ATAAVFGVGAPQARAATAAAGVEYPANRLANISELTLNEPLDVAYPDEDAAGVLLKLGTRVEGGVGPDGDIVGFSTICPHKGFPLSYSADNKTFNCPGHFSVFDPEKGGQQVWGQATQNLPQYVLRVADNGDIFAEGVDELIYGRLSNVL

SEQ ID NO: 4 - protein, 845 aa, Rhizobium sp. NT-26
MAFKRHIDRLPIIPADAKKHNVTCHFCIVGCGYHAYTWPINKQGGTDPQNNIFGVDLSEQQQAESDAWYSPSMYNVVKQDGRDVHVVIKPDHECVVNSGLGSVRGARMAETSFSEARNTQQQRLTDPLVWRYGQMQPTSWDDALDLVARVTAKIVKEKGEDALIVSAFDHGGAGGGYENTWGTGKLYFEAMKVKNIRIHNRPAYNSEVHGTRDMGVGELNNCYEDAELADTIVAVGTNALETQTNYFLNHWIPNLRGESLGKKKELMPEEPHEAGRIIIVDPRRTVTVNACEQTAGADNVLHLAINSGTDLALFNALFTYIADKGWVDRDFIDKSTLREGTARPPLYPARGVSEANPGHLSSFEDAVEGCRMSIEEAAEITGLDAAQIIKAAEWIGMPKEGGKRRRVMFGYEKGLIWGNDNYRTNGALVNLALATGNIGRPGGGVVRLGGHQEGYVRPSDAHVGRPAAYVDQLLIGGQGGVHHIWGCDHYKTTLNAHEFKRVYKKRTDMVKDAMSAAPYGDREAMVNAIVDAINQGGLFAVNVDIIPTKIGEACHVILPAATSGEMNLTSMNGERRMRLTERYMDPPGQSMPDCLIAARLANTMERVLTEMGDVGYAAQFKGFDWQTEEDAFMDGYNKNAHGGEFVTYERLSAMGTNGFQEPATGFTDGKIEGTQRLYTDGVFSTDDGKARFMDAPWRGLQAPGKQQQKDSHKYLINNGRANVVWQSAYLDQENDFVMDRFPYPFIEMNPEDMAEAGLKEGDLVEIYNDAGATQAMAYPTPTARRGETFMLFGFPTGVQGNVTSAGTNELIIPNYKQTWGNIRKISDAPRNVAHLSFKSKEYQSA

SEQ ID NO: 5 - DNA, 528 bp, Rhizobium sp. NT-26
atgtcacgttgtcaaaacatggtcgatattggccgacgccagttcctgcgtggaggcgcgctcgcggctgcgggtgcgactgccgccgtcttcggcgtcggcgcaccacaggctagagccgctaccgcggcggcaggggtcgaatatcctgccaatcgtctggcaaacatctcagaacttacgctcaatgaaccgctcgatgtcgcctatccggacgaggatgccgcaggcgttctgcttaagcttgggacccgcgtcgagggtggcgttggccctgacggcgacattgtcggcttttccacgatctgtcctcacaagggttttcctctgagctactccgccgacaacaagacgttcaactgtcctggtcacttctcggtcttcgaccctgaaaagggcggccagcaggtttggggtcaggccacgcagaacctgccgcaatacgtgctccgcgtcgccgacaatggcgacatctttgccgaaggcgtcgacgagctgatctacggccgtctgtccaacgttctataa

SEQ ID NO: 6 - DNA, 120 bp, Rhizobium sp. NT-26
atgtcacgttgtcaaaacatggtcgatattggccgacgccagttcctgcgtggaggcgcgctcgcggctgcgggtgcgactgccgccgtcttcggcgtcggcgcaccacaggctagagcc

SEQ ID NO: 7 - DNA, 408 bp, Rhizobium sp. NT-26
gctaccgcggcggcaggggtcgaatatcctgccaatcgtctggcaaacatctcagaacttacgctcaatgaaccgctcgatgtcgcctatccggacgaggatgccgcaggcgttctgcttaagcttgggacccgcgtcgagggtggcgttggccctgacggcgacattgtcggcttttccacgatctgtcctcacaagggttttcctctgagctactccgccgacaacaagacgttcaactgtcctggtcacttctcggtcttcgaccctgaaaagggcggccagcaggtttggggtcaggccacgcagaacctgccgcaatacgtgctccgcgtcgccgacaatggcgacatctttgccgaaggcgtcgacgagctgatctacggccgtctgtccaacgttctataa

SEQ ID NO: 8 - DNA, 2538 bp, Rhizobium sp. NT-26
atggccttcaaacgtcacatcgaccgtctgccgatcattcccgcggacgccaagaagcacaatgtcacctgccacttctgcatcgtcggttgcggctatcacgcctatacctggccgatcaacaaacaaggcggtacggatccacagaacaacatcttcggcgtcgacctgtctgaacagcagcaggcggaaagcgacgcctggtattcaccgtccatgtacaacgtggtcaagcaggatggccgcgacgttcatgtcgtcatcaagccagaccacgaatgtgtcgtgaactccggtctcggttcggtgcgtggcgcccgcatggcagagacgagcttctcagaggcccgcaacacccagcagcagcgcctcaccgatccgcttgtctggcgatacgggcagatgcaaccgacgagctgggacgacgcgctcgatctcgtcgctcgcgtgaccgcgaagatcgtcaaagagaagggtgaggacgccctcatcgtatcggcctttgaccatggcggtgcaggcggcggctacgagaacacctggggcacgggaaagctctatttcgaggccatgaaggtcaagaacatccgcatccacaaccgcccggcctacaattccgaggttcacggcacccgcgacatgggcgtcggcgagttgaataactgctacgaggatgccgaactggccgacacgatcgttgcggttggcaccaacgcgctggagacccagaccaactacttcctaaatcactggattccgaatctgcgcggcgaaagcctcggcaagaaaaaggagctcatgccggaggagccccatgaagcaggcaggatcattatcgtcgatccgcgccgcaccgtgacggtcaatgcctgcgagcagacggccggcgccgacaatgtcctgcatcttgctatcaattctggcacggacctcgcccttttcaacgcactcttcacctatatcgccgacaagggctgggtcgatcgcgacttcatcgacaagtcgacactgcgcgagggtacagcccgaccgccgctctatcctgcccgtggagtgtcagaggccaatccggggcatctctcgagtttcgaggacgccgtggaaggctgccgcatgtctatcgaggaggctgcggaaatcaccggtctcgacgccgcccagatcatcaaggcagccgagtggatcggcatgcccaaggaaggcggcaagcgccgccgtgtcatgttcggttacgagaagggtctgatctggggcaatgacaactaccgaaccaacggcgcgctggtgaacctcgcccttgccaccggcaatatcggccgtcccggtggcggcgtcgtacgccttggcggacaccaggaaggctatgtgcgcccctccgacgcccatgtcggccggccggcggcctatgtcgaccagttgctgatcggcggccagggcggcgttcaccacatctggggctgcgaccactacaaaacgacgctcaatgcgcatgagtttaagcgcgtctacaagaagcgcaccgacatggtgaaggacgccatgagcgctgccccctacggcgaccgcgaggccatggtcaatgccattgtcgacgcaatcaatcagggcggattgtttgccgtcaatgtcgacatcatcccgacaaaaatcggcgaagcctgtcatgttattctgcctgcggccacgtcaggcgagatgaacctcacgtcaatgaatggcgagcggcgcatgcggctgaccgaacgctatatggacccgcccggtcagtccatgccggactgcctgattgccgctcgtctcgccaacaccatggaacgcgtgctgaccgagatgggtgacgtcggctatgccgctcaattcaagggctttgactggcagacagaagaagacgccttcatggacggctacaacaagaatgcacatggcggagagttcgtcacctatgagcgcctgagtgcgatgggcaccaacggcttccaggagccggctaccggctttaccgacggcaagatcgagggcacccagcggctctataccgacggcgtattctcgaccgacgacggcaaggcgcggttcatggacgcgccatggcggggacttcaggcaccgggcaagcagcagcagaaggacagccacaagtacttgatcaacaacggccgtgccaatgtcgtctggcaatcggcgtatctcgaccaggaaaacgacttcgtcatggatcgtttcccctacccgttcatcgagatgaacccagaggacatggcggaagcaggccttaaggagggcgacctcgtcgagatttacaatgatgccggagcgacgcaggccatggcctatccgacgccgacagcccgacgtggagaaaccttcatgctgttcggttttccaaccggggttcagggcaatgtgaccagtgccgggacgaacgagttgataatcccgaactacaagcagacctggggcaatatccgcaagatttcggatgcgcccaggaacgtggctcacctttccttcaagtcgaaagaataccagtcggcttga